European Patent Specification EP 3 870 295 B1, published March 8, 2023. Title: Novel tricyclic compounds for the treatment and prophylaxis of Hepatitis B Virus disease. Applicant: F. Hoffmann-La Roche AG. The sequence listing filed with the application follows.

SEQUENCE LISTING (3 sequences)

SEQ ID NO: 1 - DNA, 20 bp, Artificial Sequence
  HBV-Forward Primer
aagaaaaaccccgcctgtaa

SEQ ID NO: 2 - DNA, 23 bp, Artificial Sequence
  HBV-Reverse Primer
cctgttctgactactgcctctcc

SEQ ID NO: 3 - DNA, 27 bp, Artificial Sequence
  HBV-Probe
cctgatgtgatgttctccatgttcagc